European Patent Application EP 4 446 341 A1, published October 16, 2024. Title: ANTIBODIES BINDING TO BCMA AND USES THEREOF. Applicant: INNOVENT BIOLOGICS (SUZHOU) CO., LTD. The sequence listing filed with the application follows.

SEQUENCE LISTING (112 sequences)

SEQ ID NO: 1 - protein, 11 aa, artificial sequence
GSISSSSYYWG

SEQ ID NO: 2 - protein, 16 aa, artificial sequence
SISYSGSTYYNPSLKS

SEQ ID NO: 3 - protein, 11 aa, artificial sequence
ARDRGDTILDV

SEQ ID NO: 4 - protein, 26 aa, artificial sequence
QLQLQESGPGLVKPSETLSLTCTVSG

SEQ ID NO: 5 - protein, 14 aa, artificial sequence
WIRQPPGKGLEWIG

SEQ ID NO: 6 - protein, 30 aa, artificial sequence
RVTISVDTSKNQFSLKLSSVTAADTAVYYC

SEQ ID NO: 7 - protein, 11 aa, artificial sequence
WGQGTMVTVSS

SEQ ID NO: 8 - DNA, 357 bp, artificial sequence
  source 1..357: mol_type = other DNA
cagctgcagctgcaggagtcgggcccaggactggtgaagccttcggagaccctgtccctcacctgcactgtctctggtggctccatcagcagtagtagttactactggggctggatccgccagcccccagggaaggggctggagtggattgggagtatctcctatagtgggagcacctactacaacccgtccctcaagagtcgagtcaccatatccgtagacacgtccaagaaccagttctccctgaagctgagttctgtgaccgccgcagacacggcggtgtactactgcgccagagatcgtggagacaccatactagacgtatggggtcagggtacaatggtcaccgtctcctca

SEQ ID NO: 9 - protein, 119 aa, artificial sequence
QLQLQESGPGLVKPSETLSLTCTVSGGSISSSSYYWGWIRQPPGKGLEWIGSISYSGSTYYNPSLKSRVTISVDTSKNQFSLKLSSVTAADTAVYYCARDRGDTILDVWGQGTMVTVSS

SEQ ID NO: 10 - protein, 11 aa, artificial sequence
RASQSISRYLN

SEQ ID NO: 11 - protein, 7 aa, artificial sequence
AASSLQS

SEQ ID NO: 12 - protein, 8 aa, artificial sequence
QQKYFDIT

SEQ ID NO: 13 - protein, 23 aa, artificial sequence
DIQMTQSPSSLSASVGDRVTITC

SEQ ID NO: 14 - protein, 15 aa, artificial sequence
WYQQKPGKAPKLLIY

SEQ ID NO: 15 - protein, 32 aa, artificial sequence
GVPSRFSGSGSGTDFTLTISSLQPEDFATYYC

SEQ ID NO: 16 - protein, 10 aa, artificial sequence
FGGGTKVEIK

SEQ ID NO: 17 - DNA, 318 bp, artificial sequence
  source 1..318: mol_type = other DNA
gacatccagatgacccagtctccatcctccctgtctgcatctgtaggagacagagtcaccatcacttgccgggcaagtcagagcattagcagatatttaaattggtatcagcagaaaccagggaaagcccctaagctcctgatctatgctgcatccagtttgcaaagtggggtcccatcaaggttcagtggcagtggatctgggacagatttcactctcaccatcagcagtctgcaacctgaagattttgcaacttactactgtcagcaaaaatacttcgacatcacttttggcggagggaccaaggttgagatcaaa

SEQ ID NO: 18 - protein, 106 aa, artificial sequence
DIQMTQSPSSLSASVGDRVTITCRASQSISRYLNWYQQKPGKAPKLLIYAASSLQSGVPSRFSGSGSGTDFTLTISSLQPEDFATYYCQQKYFDITFGGGTKVEIK

SEQ ID NO: 19 - protein, 11 aa, artificial sequence
GSIVSSSYYWT

SEQ ID NO: 20 - protein, 16 aa, artificial sequence
SISIAGSTYYNPSLKS

SEQ ID NO: 21 - protein, 11 aa, artificial sequence
ARDRGDTILDV

SEQ ID NO: 22 - protein, 26 aa, artificial sequence
QLQLQESGPGLVKPSETLSLTCTVSG

SEQ ID NO: 23 - protein, 14 aa, artificial sequence
WIRQPPGKGLEWIG

SEQ ID NO: 24 - protein, 30 aa, artificial sequence; identical to SEQ ID NO: 6

SEQ ID NO: 25 - protein, 11 aa, artificial sequence
WGQGTMVTVSS

SEQ ID NO: 26 - DNA, 357 bp, artificial sequence
  source 1..357: mol_type = other DNA
cagctgcagctgcaggagtcgggcccaggactggtgaagccttcggagaccctgtccctcacctgcactgtctctggtggctccatcgtcagtagtagttactactggacctggatccgccagcccccagggaaggggctggagtggattgggagtatctccatagcagggagcacctactacaacccgtccctcaagagtcgagtcaccatatccgtagacacgtccaagaaccagttctccctgaagctgagttctgtgaccgccgcagacacggcggtgtactactgcgccagagatcgtggagacaccatactagacgtatggggtcagggtacaatggtcaccgtctcctca

SEQ ID NO: 27 - protein, 119 aa, artificial sequence
QLQLQESGPGLVKPSETLSLTCTVSGGSIVSSSYYWTWIRQPPGKGLEWIGSISIAGSTYYNPSLKSRVTISVDTSKNQFSLKLSSVTAADTAVYYCARDRGDTILDVWGQGTMVTVSS

SEQ ID NO: 28 - protein, 11 aa, artificial sequence
RASQSISRYLN

SEQ ID NO: 29 - protein, 7 aa, artificial sequence
AASSLQS

SEQ ID NO: 30 - protein, 8 aa, artificial sequence
QQKYFDIT

SEQ ID NO: 31 - protein, 23 aa, artificial sequence
DIQMTQSPSSLSASVGDRVTITC

SEQ ID NO: 32 - protein, 15 aa, artificial sequence
WYQQKPGKAPKLLIY

SEQ ID NO: 33 - protein, 32 aa, artificial sequence; identical to SEQ ID NO: 15

SEQ ID NO: 34 - protein, 10 aa, artificial sequence
FGGGTKVEIK

SEQ ID NO: 35 - DNA, 318 bp, artificial sequence; identical to SEQ ID NO: 17
  source 1..318: mol_type = other DNA

SEQ ID NO: 36 - protein, 106 aa, artificial sequence; identical to SEQ ID NO: 18

SEQ ID NO: 37 - protein, 11 aa, artificial sequence
GSIVSSSYYWT

SEQ ID NO: 38 - protein, 16 aa, artificial sequence
SISIAGSTYYNPSLKS

SEQ ID NO: 39 - protein, 11 aa, artificial sequence
ARDRGDQILDV

SEQ ID NO: 40 - protein, 26 aa, artificial sequence
QLQLQESGPGLVKPSETLSLTCTVSG

SEQ ID NO: 41 - protein, 14 aa, artificial sequence
WIRQPPGKGLEWIG

SEQ ID NO: 42 - protein, 30 aa, artificial sequence; identical to SEQ ID NO: 6

SEQ ID NO: 43 - protein, 11 aa, artificial sequence
WSQGTMVTVSS

SEQ ID NO: 44 - DNA, 357 bp, artificial sequence
  source 1..357: mol_type = other DNA
cagctgcagctgcaggagtcgggcccaggactggtgaagccttcggagaccctgtccctcacctgcactgtctctggtggctccatcgtcagtagtagttactactggacctggatccgccagcccccagggaaggggctggagtggattgggagtatctccatagcagggagcacctactacaacccgtccctcaagagtcgagtcaccatatccgtagacacgtccaagaaccagttctccctgaagctgagttctgtgaccgccgcagacacggcggtgtactactgcgccagagatcgtggagaccagattctagacgtatggagtcagggtacaatggtcaccgtctcctca

SEQ ID NO: 45 - protein, 119 aa, artificial sequence
QLQLQESGPGLVKPSETLSLTCTVSGGSIVSSSYYWTWIRQPPGKGLEWIGSISIAGSTYYNPSLKSRVTISVDTSKNQFSLKLSSVTAADTAVYYCARDRGDQILDVWSQGTMVTVSS

SEQ ID NO: 46 - protein, 11 aa, artificial sequence
RASQSISRYLN

SEQ ID NO: 47 - protein, 7 aa, artificial sequence
AASSLQS

SEQ ID NO: 48 - protein, 8 aa, artificial sequence
QQKYFDIT

SEQ ID NO: 49 - protein, 23 aa, artificial sequence
DIQMTQSPSSLSASVGDRVTITC

SEQ ID NO: 50 - protein, 15 aa, artificial sequence
WYQQKPGKAPKLLIY

SEQ ID NO: 51 - protein, 32 aa, artificial sequence; identical to SEQ ID NO: 15

SEQ ID NO: 52 - protein, 10 aa, artificial sequence
FGGGTKVEIK

SEQ ID NO: 53 - DNA, 318 bp, artificial sequence; identical to SEQ ID NO: 17
  source 1..318: mol_type = other DNA

SEQ ID NO: 54 - protein, 106 aa, artificial sequence; identical to SEQ ID NO: 18

SEQ ID NO: 55 - protein, 9 aa, artificial sequence
GTFSNYAIS

SEQ ID NO: 56 - protein, 17 aa, artificial sequence
GIIPIFGTANYAQKFQG

SEQ ID NO: 57 - protein, 14 aa, artificial sequence
ARGRGYYSSWLFDI

SEQ ID NO: 58 - protein, 26 aa, artificial sequence
QVQLVQSGAEVKKPGSSVKVSCKASG

SEQ ID NO: 59 - protein, 14 aa, artificial sequence
WVRQAPGQGLEWMG

SEQ ID NO: 60 - protein, 30 aa, artificial sequence
RVTITADESTSTAYMELSSLRSEDTAVYYC

SEQ ID NO: 61 - protein, 11 aa, artificial sequence
WGQGTMVTVSS

SEQ ID NO: 62 - DNA, 363 bp, artificial sequence
  source 1..363: mol_type = other DNA
caggtgcagctggtgcagtctggggctgaggtgaagaagcctgggtcctcggtgaaggtctcctgcaaggcttctggaggcaccttcagcaactatgctatcagctgggtgcgacaggcccctggacaagggcttgagtggatgggagggatcatccctatctttggtacagcaaactacgcacagaagttccagggcagagtcacgattaccgcggacgaatccacgagcacagcctacatggagctgagcagcctgagatctgaggacacggcggtgtactactgcgccagaggcaggggatactactcaagctggctattcgacatatggggtcagggtacaatggtcaccgtctcctca

SEQ ID NO: 63 - protein, 121 aa, artificial sequence
QVQLVQSGAEVKKPGSSVKVSCKASGGTFSNYAISWVRQAPGQGLEWMGGIIPIFGTANYAQKFQGRVTITADESTSTAYMELSSLRSEDTAVYYCARGRGYYSSWLFDIWGQGTMVTVSS

SEQ ID NO: 64 - protein, 11 aa, artificial sequence
QASQDITNYLN

SEQ ID NO: 65 - protein, 7 aa, artificial sequence
DASNLET

SEQ ID NO: 66 - protein, 8 aa, artificial sequence
QQAFDLIT

SEQ ID NO: 67 - protein, 23 aa, artificial sequence
DIQMTQSPSSLSASVGDRVTITC

SEQ ID NO: 68 - protein, 15 aa, artificial sequence
WYQQKPGKAPKLLIY

SEQ ID NO: 69 - protein, 32 aa, artificial sequence
GVPSRFSGSGSGTDFTFTISSLQPEDIATYYC

SEQ ID NO: 70 - protein, 10 aa, artificial sequence
FGGGTKVEIK

SEQ ID NO: 71 - DNA, 318 bp, artificial sequence
  source 1..318: mol_type = other DNA
gacatccagatgacccagtctccatcctccctgtctgcatctgtaggagacagagtcaccatcacttgccaggcgagtcaggacattaccaactatttaaattggtatcagcagaaaccagggaaagcccctaagctcctgatctacgatgcatccaatttggaaacaggggtcccatcaaggttcagtggaagtggatctgggacagattttactttcaccatcagcagcctgcagcctgaagatattgcaacatattactgtcagcaggccttcgacctcatcacttttggcggagggaccaaggttgagatcaaa

SEQ ID NO: 72 - protein, 106 aa, artificial sequence
DIQMTQSPSSLSASVGDRVTITCQASQDITNYLNWYQQKPGKAPKLLIYDASNLETGVPSRFSGSGSGTDFTFTISSLQPEDIATYYCQQAFDLITFGGGTKVEIK

SEQ ID NO: 73 - protein, 9 aa, artificial sequence
GTFSNDVIS

SEQ ID NO: 74 - protein, 17 aa, artificial sequence
VIIPIFGIANYAQKFQG

SEQ ID NO: 75 - protein, 14 aa, artificial sequence
ARGRGYYSSWLLDI

SEQ ID NO: 76 - protein, 26 aa, artificial sequence
QVQLVQSGAEVKKPGSSVKVSCKASG

SEQ ID NO: 77 - protein, 14 aa, artificial sequence
WVRQAPGQGLEWMG

SEQ ID NO: 78 - protein, 30 aa, artificial sequence; identical to SEQ ID NO: 60

SEQ ID NO: 79 - protein, 11 aa, artificial sequence
WGQGTMVTVSS

SEQ ID NO: 80 - DNA, 363 bp, artificial sequence
  source 1..363: mol_type = other DNA
caggtgcagctggtgcagtctggggctgaggtgaagaagcctgggtcctcggtgaaggtctcctgcaaggcttctggaggcaccttcagcaacgacgtcatcagctgggtgcgacaggcccctggacaagggcttgagtggatgggagtcatcatccctatcttcggtatagcaaactacgcacagaagttccagggcagagtcacgattaccgcggacgaatccacgagcacagcctacatggagctgagcagcctgagatctgaggacacggcggtgtactactgcgccagaggcaggggatactactcaagctggcttttggacatatggggtcagggtacaatggtcaccgtctcctca

SEQ ID NO: 81 - protein, 121 aa, artificial sequence
QVQLVQSGAEVKKPGSSVKVSCKASGGTFSNDVISWVRQAPGQGLEWMGVIIPIFGIANYAQKFQGRVTITADESTSTAYMELSSLRSEDTAVYYCARGRGYYSSWLLDIWGQGTMVTVSS

SEQ ID NO: 82 - protein, 11 aa, artificial sequence
QASQDITNYLN

SEQ ID NO: 83 - protein, 7 aa, artificial sequence
DASNLET

SEQ ID NO: 84 - protein, 8 aa, artificial sequence
QQAFDLIT

SEQ ID NO: 85 - protein, 23 aa, artificial sequence
DIQMTQSPSSLSASVGDRVTITC

SEQ ID NO: 86 - protein, 15 aa, artificial sequence
WYQQKPGKAPKLLIY

SEQ ID NO: 87 - protein, 32 aa, artificial sequence; identical to SEQ ID NO: 69

SEQ ID NO: 88 - protein, 10 aa, artificial sequence
FGGGTKVEIK

SEQ ID NO: 89 - DNA, 318 bp, artificial sequence; identical to SEQ ID NO: 71
  source 1..318: mol_type = other DNA

SEQ ID NO: 90 - protein, 106 aa, artificial sequence; identical to SEQ ID NO: 72

SEQ ID NO: 91 - protein, 9 aa, artificial sequence
GTFSNDVIS

SEQ ID NO: 92 - protein, 17 aa, artificial sequence
VIIPIFGIANYAQKFQG

SEQ ID NO: 93 - protein, 14 aa, artificial sequence
ARGRGYYSSWLHDI

SEQ ID NO: 94 - protein, 26 aa, artificial sequence
QVQLVQSGAEVKKPGSSVKVSCKASG

SEQ ID NO: 95 - protein, 14 aa, artificial sequence
WVRQAPGQGLEWMG

SEQ ID NO: 96 - protein, 30 aa, artificial sequence; identical to SEQ ID NO: 60

SEQ ID NO: 97 - protein, 11 aa, artificial sequence
WGQGTMVTVSS

SEQ ID NO: 98 - DNA, 363 bp, artificial sequence
  source 1..363: mol_type = other DNA
caggtgcagctggtgcagtctggggctgaggtgaagaagcctgggtcctcggtgaaggtctcctgcaaggcttctggaggcaccttcagcaacgacgtcatcagctgggtgcgacaggcccctggacaagggcttgagtggatgggagtcatcatccctatcttcggtatagcaaactacgcacagaagttccagggcagagtcacgattaccgcggacgaatccacgagcacagcctacatggagctgagcagcctgagatctgaggacacggcggtgtactactgcgccagaggcaggggatactactcaagctggctgcatgacatatggggtcagggtacaatggtcaccgtctcctca

SEQ ID NO: 99 - protein, 121 aa, artificial sequence
QVQLVQSGAEVKKPGSSVKVSCKASGGTFSNDVISWVRQAPGQGLEWMGVIIPIFGIANYAQKFQGRVTITADESTSTAYMELSSLRSEDTAVYYCARGRGYYSSWLHDIWGQGTMVTVSS

SEQ ID NO: 100 - protein, 11 aa, artificial sequence
QASQDITNYLN

SEQ ID NO: 101 - protein, 7 aa, artificial sequence
DASNLET

SEQ ID NO: 102 - protein, 8 aa, artificial sequence
QQAFDLIT

SEQ ID NO: 103 - protein, 23 aa, artificial sequence
DIQMTQSPSSLSASVGDRVTITC

SEQ ID NO: 104 - protein, 15 aa, artificial sequence
WYQQKPGKAPKLLIY

SEQ ID NO: 105 - protein, 32 aa, artificial sequence; identical to SEQ ID NO: 69

SEQ ID NO: 106 - protein, 10 aa, artificial sequence
FGGGTKVEIK

SEQ ID NO: 107 - DNA, 318 bp, artificial sequence
  source 1..318: mol_type = other DNA
gacatccagatgacccagtctccatcctccctgtctgcatctgtaggagacagagtcaccatcacttgccaggcgagtcaggacattaccaactatttaaattggtatcagcagaaaccagggaaagcccctaagctcctgatctacgatgcatccaatttggaaacaggggtcccatcaaggttcagtggaagtggatctgggacagattttactttcaccatcagcagcctgcagcctgaagatattgcaacatattactgtcagcaggccttcgacctcatcactttcggcggagggaccaaggtggagatcaaa

SEQ ID NO: 108 - protein, 106 aa, artificial sequence; identical to SEQ ID NO: 72

SEQ ID NO: 109 - protein, 184 aa, artificial sequence
MLQMAGQCSQNEYFDSLLHACIPCQLRCSSNTPPLTCQRYCNASVTNSVKGTNAILWTCLGLSLIISLAVFVLMFLLRKINSEPLKDEFKNTGSGLLGMANIDLEKSRTGDEIILPRGLEYTVEECTCEDCIKSKPKVDSDHCFPLPAMEEGATILVTTKTNDYCKSLPAALSATEIEKSISAR

SEQ ID NO: 110 - protein, 330 aa, artificial sequence [sequence omitted]

SEQ ID NO: 111 - protein, 330 aa, artificial sequence
ASTKGPSVFPLAPSSKSTSGGTAALGCLVKDYFPEPVTVSWNSGALTSGVHTFPAVLQSSGLYSLSSVVTVPSSSLGTQTYICNVNHKPSNTKVDKKVEPKSCDKTHTCPPCPAPELLGGPSVFLFPPKPKDTLMISRTPEVTCVVVDVSHEDPEVKFNWYVDGVEVHNAKTKPREEQYNSTYRVVSVLTVLHQDWLNGKEYKCKVSNKALGAPIEKTISKAKGQPREPQVYTLPPSRDELTKNQVSLTCLVKGFYPSDIAVEWESNGQPENNYKTTPPVLDSDGSFFLYSKLTVDKSRWQQGNVFSCSVMHEALHNHYTQKSLSLSPGK

SEQ ID NO: 112 - protein, 107 aa, artificial sequence [sequence omitted]